European Patent Specification EP 3 841 107 B1, published June 28, 2023. Title: SOLUTION PHASE ROUTES FOR WNT HEXAPEPTIDES. Applicant: WntResearch AB. The sequence listing filed with the application follows.

SEQUENCE LISTING (15 sequences)

SEQ ID NO: 1 - protein, 6 aa, Artificial Sequence
  MOD_RES 1: Formyl-methionine
  Peptide
MDGCEL

SEQ ID NO: 2 - protein, 6 aa, Artificial Sequence
  MOD_RES 1: (Tert-Butoxycarbonyl)-methionine
  Synthetic peptide
  MOD_RES 2: Aspartic acid tert-butylester
  MOD_RES 4: Trityl-cystein
  MOD_RES 5: Glutamic acid tert-butylester
  MOD_RES 6: Leucine tert-butylester
MDGCEL

SEQ ID NO: 3 - protein, 5 aa, Artificial Sequence
  MOD_RES 1: (Fluorenylmethoxycarbonyl)-aspartic acid tert-butylester
  Synthetic peptide
  MOD_RES 3: Trityl-cystein
  MOD_RES 4: Glutamic acid tert-butylester
  MOD_RES 5: Leucine tert-butylester
DGCEL

SEQ ID NO: 4 - protein, 6 aa, Artificial Sequence
  MOD_RES 1: Formyl-methionine
  Synthetic peptide
  MOD_RES 2: Aspartic acid tert-butylester
  MOD_RES 4: Trityl-cystein
  MOD_RES 5: Glutamic acid tert-butylester
  MOD_RES 6: Leucine tert-butylester
MDGCEL

SEQ ID NO: 5 - protein, 4 aa, Artificial Sequence
  Synthetic peptide
  MOD_RES 2: Cysteine acetonide
  MOD_RES 3: Glutamic acid tert-butylester
  MOD_RES 4: Leucine tert-butylester
GCEL

SEQ ID NO: 6 - protein, 4 aa, Artificial Sequence
  MOD_RES 1: (Fluorenylmethoxycarbonyl)-glycine
  Synthetide peptide
  MOD_RES 2: Trityl-cystein
  MOD_RES 3: Glutamic acid tert-butylester
  MOD_RES 4: Leucine tert-butylester
GCEL

SEQ ID NO: 7 - protein, 4 aa, Artificial Sequence
  MOD_RES 1: (Fluorenylmethoxycarbonyl)-glycine
  Synthetic peptide
  MOD_RES 2: Trityl-cystein
  MOD_RES 3: Glutamic acid tert-butylester
  MOD_RES 4: Leucine tert-butylester
GCEL

SEQ ID NO: 8 - protein, 4 aa, Artificial Sequence
  Synthetic peptide
GCEL

SEQ ID NO: 9 - protein, 5 aa, Artificial Sequence
  MOD_RES 1: (Fluorenylmethoxycarbonyl)-aspartic acid tert-butylester
  Synthetic sequence
  MOD_RES 3: Trityl-cystein
  MOD_RES 4: Glutamic acid tert-butylester
  MOD_RES 5: Leucine-methylester
DGCEL

SEQ ID NO: 10 - protein, 5 aa, Artificial Sequence
  MOD_RES 1: (Fluorenylmethoxycarbonyl)-aspartic acid tert-butylester
  Syntheti peptide
  MOD_RES 3: Trityl-cystein
  MOD_RES 4: Glutamic acid tert-butylester
  MOD_RES 5: Leucine-methylester
DGCEL

SEQ ID NO: 11 - protein, 5 aa, Artificial Sequence
  Synthetic peptide
MDGCC

SEQ ID NO: 12 - protein, 4 aa, Artificial Sequence
  MOD_RES 1: Carboxybenzyl-methionine
  Synthetic peptide
  MOD_RES 2: Aspartic acid benzylester
  MOD_RES 4: Benzylcysteine
MDGC

SEQ ID NO: 13 - protein, 6 aa, Artificial Sequence
  MOD_RES 1: Carboxybenzyl-methionine
  Synthetic peptide
  MOD_RES 2: Aspartic acid benzylester
  MOD_RES 4: Benzylcysteine
  MOD_RES 5: Glutamic acid benzylester
  MOD_RES 6: Leucine benzylester
MDGCEL

SEQ ID NO: 14 - protein, 6 aa, Artificial Sequence
  Synthetic peptide
MDGCEL

SEQ ID NO: 15 - protein, 6 aa, Artificial Sequence
  MOD_RES 1: (Tert-Butoxycarbonyl)-methionine
  Synthetic peptide
  MOD_RES 2: Aspartic acid tert-butylester
  MOD_RES 4: Trityl-cystein
  MOD_RES 5: Glutamic acid tert-butylester
  MOD_RES 6: Leucine tert-butylester
MDGCEL